European Patent Application EP 4 752 224 A1, published June 3, 2026. Title: AAV mutant with tropism for brain. Applicant: タカラバイオ株式会社. The sequence listing filed with the application follows.

SEQUENCE LISTING (12 sequences)

SEQ ID NO: 1 - protein, 7 aa, Synthetic construct
ETGHGYV

SEQ ID NO: 2 - protein, 7 aa, Synthetic construct
ETGHGFV

SEQ ID NO: 3 - protein, 7 aa, Synthetic construct
ETGHAWV

SEQ ID NO: 4 - protein, 7 aa, Synthetic construct
ETGHGWA

SEQ ID NO: 5 - DNA, 49 bp, Synthetic construct
  source 1..49: mol_type = other DNA
taaggatccgcacnnnnnnnnnnnnnnnctggggatccacgggtggcat

SEQ ID NO: 6 - DNA, 21 bp, Synthetic construct
  source 1..21: mol_type = other DNA
atgccacccgtggatccccag

SEQ ID NO: 7 - DNA, 59 bp, Synthetic construct
  source 1..59: mol_type = other DNA
gtctcgtgggctcggagatgtgtataagagacagccgatttcaaggaggatggcaacat

SEQ ID NO: 8 - DNA, 58 bp, Synthetic construct
  source 1..58: mol_type = other DNA
tcgtcggcagcgtcagatgtgtataagagacaggtgggcactggagtggcaacttcca

SEQ ID NO: 9 - protein, 735 aa, Adeno-associated virus type 2 [sequence omitted]

SEQ ID NO: 10 - protein, 735 aa, Synthetic construct
MAADGYLPDWLEDTLSEGIRQWWKLKPGPPPPKPAERHKDDSRGLVLPGYKYLGPFNGLDKGEPVNEADAAALEHDKAYDRQLDSGDNPYLKYNHADAEFQERLKEDTSFGGNLGRAVFQAKKRVLEPLGLVEEPVKTAPGKKRPVEHSPVEPDSSSGTGKAGQQPARKRLNFGQTGDADSVPDPQPLGQPPAAPSGLGTNTMATGSGAPMADNNEGADGVGNSSGNWHCDSTWMGDRVITTSTRTWALPTYNNHLYKQISSQSGASNDNHYFGYSTPWGYFDFNRFHCHFSPRDWQRLINNNWGFRPKRLNFKLFNIQVKEVTQNDGTTTIANNLTSTVQVFTDSEYQLPYVLGSAHQGCLPPFPADVFMVPQYGYLTLNNGSQAVGRSSFYCLEYFPSQMLRTGNNFTFSYTFEDVPFHSSYAHSQSLDRLMNPLIDQYLYYLSRTNTPSGTTTQSRLQFSQAGASDIRDQSRNWLPGPCYRQQRVSKTSADNNNSEYSWTGATKYHLNGRDSLVNPGPAMASHKDDEEKFFPQSGVLIFGKQGSEKTNVDIEKVMITDEEEIRTTNPVATEQYGSVSTNLQRGQRQAATADVNTQGVLPGMVWQDRDVYLQGPIWAKIPHTDGHFHPSPLMGGFGLKHPPPQILIKNTPVPANPSTTFSAAKFASFITQYSTGQVSVEIEWELQKENSKRWNPEIQYTSNYNKSVNVDFTVDTNGVYSEPRPIGTRYLTRNL

SEQ ID NO: 11 - protein, 744 aa, Synthetic construct
MAADGYLPDWLEDTLSEGIRQWWKLKPGPPPPKPAERHKDDSRGLVLPGYKYLGPFNGLDKGEPVNEADAAALEHDKAYDRQLDSGDNPYLKYNHADAEFQERLKEDTSFGGNLGRAVFQAKKRVLEPLGLVEEPVKTAPGKKRPVEHSPVEPDSSSGTGKAGQQPARKRLNFGQTGDADSVPDPQPLGQPPAAPSGLGTNTMATGSGAPMADNNEGADGVGNSSGNWHCDSTWMGDRVITTSTRTWALPTYNNHLYKQISSQSGASNDNHYFGYSTPWGYFDFNRFHCHFSPRDWQRLINNNWGFRPKRLNFKLFNIQVKEVTQNDGTTTIANNLTSTVQVFTDSEYQLPYVLGSAHQGCLPPFPADVFMVPQYGYLTLNNGSQAVGRSSFYCLEYFPSQMLRTGNNFTFSYTFEDVPFHSSYAHSQSLDRLMNPLIDQYLYYLSRTNTPSGTTTQSRLQFSQAGASDIRDQSRNWLPGPCYRQQRVSKTSADNNNSEYSWTGATKYHLNGRDSLVNPGPAMASHKDDEEKFFPQSGVLIFGKQGSEKTNVDIEKVMITDEEEIRTTNPVATEQYGSVSTNLQRGNRGETGHGWVAQAATADVNTQGVLPGMVWQDRDVYLQGPIWAKIPHTDGHFHPSPLMGGFGLKHPPPQILIKNTPVPANPSTTFSAAKFASFITQYSTGQVSVEIEWELQKENSKRWNPEIQYTSNYNKSVNVDFTVDTNGVYSEPRPIGTRYLTRNL

SEQ ID NO: 12 - protein, 744 aa, Synthetic construct
MAADGYLPDWLEDTLSEGIRQWWKLKPGPPPPKPAERHKDDSRGLVLPGYKYLGPFNGLDKGEPVNEADAAALEHDKAYDRQLDSGDNPYLKYNHADAEFQERLKEDTSFGGNLGRAVFQAKKRVLEPLGLVEEPVKTAPGKKRPVEHSPVEPDSSSGTGKAGQQPARKRLNFGQTGDADSVPDPQPLGQPPAAPSGLGTNTMATGSGAPMADNNEGADGVGNSSGNWHCDSTWMGDRVITTSTRTWALPTYNNHLYKQISSQSGASNDNHYFGYSTPWGYFDFNRFHCHFSPRDWQRLINNNWGFRPKRLNFKLFNIQVKEVTQNDGTTTIANNLTSTVQVFTDSEYQLPYVLGSAHQGCLPPFPADVFMVPQYGYLTLNNGSQAVGRSSFYCLEYFPSQMLRTGNNFTFSYTFEDVPFHSSYAHSQSLDRLMNPLIDQYLYYLSRTNTPSGTTTQSRLQFSQAGASDIRDQSRNWLPGPCYRQQRVSKTSADNNNSEYSWTGATKYHLNGRDSLVNPGPAMASHKDDEEKFFPQSGVLIFGKQGSEKTNVDIEKVMITDEEEIRTTNPVATEQYGSVSTNLQRGNRGETGHGYVAQAATADVNTQGVLPGMVWQDRDVYLQGPIWAKIPHTDGHFHPSPLMGGFGLKHPPPQILIKNTPVPANPSTTFSAAKFASFITQYSTGQVSVEIEWELQKENSKRWNPEIQYTSNYNKSVNVDFTVDTNGVYSEPRPIGTRYLTRNL